European Patent Application EP 4 286 412 A1, published December 6, 2023. Title: Novel binding molecule and use thereof. Applicant: Good T Cells, Inc. The sequence listing filed with the application follows.

SEQUENCE LISTING (54 sequences)

SEQ ID NO: 1 - protein, 759 aa, Homo sapiens
GPRAPCAAACTCAGDSLDCGGRGLAALPGDLPSWTRSLNLSYNKLSEIDPAGFEDLPNLQEVYLNNNELTAVPSLGAASSHVVSLFLQHNKIRSVEGSQLKAYLSLEVLDLSLNNITEVRNTCFPHGPPIKELNLAGNRIGTLELGAFDGLSRSLLTLRLSKNRITQLPVRAFKLPRLTQLDLNRNRIRLIEGLTFQGLNSLEVLKLQRNNISKLTDGAFWGLSKMHVLHLEYNSLVEVNSGSLYGLTALHQLHLSNNSIARIHRKGWSFCQKLHELVLSFNNLTRLDEESLAELSSLSVLRLSHNSISHIAEGAFKGLRSLRVLDLDHNEISGTIEDTSGAFSGLDSLSKLTLFGNKIKSVAKRAFSGLEGLEHLNLGGNAIRSVQFDAFVKMKNLKELHISSDSFLCDCQLKWLPPWLIGRMLQAFVTATCAHPESLKGQSIFSVPPESFVCDDFLKPQIITQPETTMAMVGKDIRFTCSAASSSSSPMTFAWKKDNEVLTNADMENFVHVHAQDGEVMEYTTILHLRQVTFGHEGRYQCVITNHFGSTYSHKARLTVNVLPSFTKTPHDITIRTTTVARLECAATGHPNPQIAWQKDGGTDFPAARERRMHVMPDDDVFFITDVKIDDAGVYSCTAQNSAGSISANATLTVLETPSLVVPLEDRVVSVGETVALQCKATGNPPPRITWFKGDRPLSLTERHHLTPDNQLLVVQNVVAEDAGRYTCEMSNTLGTERAHSQLSVLPAAGCRKDGTTVG

SEQ ID NO: 2 - DNA, 2397 bp, Homo sapiens
ggcccgcgggcgccctgcgcggccgcctgcacttgcgctggggactcgctggactgcggtgggcgcgggctggctgcgttgcccggggacctgccctcctggacgcggagcctaaacctgagttacaacaaactctctgagattgaccctgctggttttgaggacttgccgaacctacaggaagtgtacctcaataataatgagttgacagcggtaccatccctgggcgctgcttcatcacatgtcgtctctctctttctgcagcacaacaagattcgcagcgtggaggggagccagctgaaggcctacctttccttagaagtgttagatctgagtttgaacaacatcacggaagtgcggaacacctgctttccacacggaccgcctataaaggagctcaacctggcaggcaatcggattggcaccctggagttgggagcatttgatggtctgtcacggtcgctgctaactcttcgcctgagcaaaaacaggatcacccagcttcctgtaagagcattcaagctacccaggctgacacaactggacctcaatcggaacaggattcggctgatagagggcctcaccttccaggggctcaacagcttggaggtgctgaagcttcagcgaaacaacatcagcaaactgacagatggggccttctggggactgtccaagatgcatgtgctgcacctggagtacaacagcctggtagaagtgaacagcggctcgctctacggcctcacggccctgcatcagctccacctcagcaacaattccatcgctcgcattcaccgcaagggctggagcttctgccagaagctgcatgagttggtcctgtccttcaacaacctgacacggctggacgaggagagcctggccgagctgagcagcctgagtgtcctgcgtctcagccacaattccatcagccacattgcggagggtgccttcaagggactcaggagcctgcgagtcttggatctggaccataacgagatttcgggcacaatagaggacacgagcggcgccttctcagggctcgacagcctcagcaagctgactctgtttggaaacaagatcaagtctgtggctaagagagcattctcggggctggaaggcctggagcacctgaaccttggagggaatgcgatcagatctgtccagtttgatgcctttgtgaagatgaagaatcttaaagagctccatatcagcagcgacagcttcctgtgtgactgccagctgaagtggctgcccccgtggctaattggcaggatgctgcaggcctttgtgacagccacctgtgcccacccagaatcactgaagggtcagagcattttctctgtgccaccagagagtttcgtgtgcgatgacttcctgaagccacagatcatcacccagccagaaaccaccatggctatggtgggcaaggacatccggtttacatgctcagcagccagcagcagcagctcccccatgacctttgcctggaagaaagacaatgaagtcctgaccaatgcagacatggagaactttgtccacgtccacgcgcaggacggggaagtgatggagtacaccaccatcctgcacctccgtcaggtcactttcgggcacgagggccgctaccaatgtgtcatcaccaaccactttggctccacctattcacataaggccaggctcaccgtgaatgtgttgccatcattcaccaaaacgccccacgacataaccatccggaccaccaccgtggcccgcctcgaatgtgctgccacaggtcacccaaaccctcagattgcctggcagaaggatggaggcacggatttccccgctgcccgtgagcgacgcatgcatgtcatgccggatgacgacgtgtttttcatcactgatgtgaaaatagatgacgcaggggtttacagctgtactgctcagaactcagccggttctatttcagctaatgccaccctgactgtcctagagaccccatccttggtggtccccttggaagaccgtgtggtatctgtgggagaaacagtggccctccaatgcaaagccacggggaaccctccgccccgcatcacctggttcaagggggaccgcccgctgagcctcactgagcggcaccacctgacccctgacaaccagctcctggtggttcagaacgtggtggcagaggatgcgggccgatatacctgtgagatgtccaacaccctgggcacggagcgagctcacagccagctgagcgtcctgcccgcagcaggctgcaggaaggatgggaccacggtaggcatcttcaccattgctgtcgtgagcagcatcgtcctgacgtcactggtctgggtgtgcatcatctaccagaccaggaagaagagtgaagagtacagtgtcaccaacacagatgaaaccgtc

SEQ ID NO: 3 - protein, 761 aa, Mus musculus
QAGPRAPCAAACTCAGDSLDCSGRGLATLPRDLPSWTRSLNLSYNRLSEIDSAAFEDLTNLQEVYLNSNELTAIPSLGAASIGVVSLFLQHNKILSVDGSQLKSYLSLEVLDLSSNNITEIRSSCFPNGLRIRELNLASNRISILESGAFDGLSRSLLTLRLSKNRITQLPVKAFKLPRLTQLDLNRNRIRLIEGLTFQGLDSLEVLRLQRNNISRLTDGAFWGLSKMHVLHLEYNSLVEVNSGSLYGLTALHQLHLSNNSISRIQRDGWSFCQKLHELILSFNNLTRLDEESLAELSSLSILRLSHNAISHIAEGAFKGLKSLRVLDLDHNEISGTIEDTSGAFTGLDNLSKLTLFGNKIKSVAKRAFSGLESLEHLNLGENAIRSVQFDAFAKMKNLKELYISSESFLCDCQLKWLPPWLMGRMLQAFVTATCAHPESLKGQSIFSVLPDSFVCDDFPKPQIITQPETTMAVVGKDIRFTCSAASSSSSPMTFAWKKDNEVLANADMENFAHVRAQDGEVMEYTTILHLRHVTFGHEGRYQCIITNHFGSTYSHKARLTVNVLPSFTKIPHDIAIRTGTTARLECAATGHPNPQIAWQKDGGTDFPAARERRMHVMPDDDVFFITDVKIDDMGVYSCTAQNSAGSVSANATLTVLETPSLAVPLEDRVVTVGETVAFQCKATGSPTPRITWLKGGRPLSLTERHHFTPGNQLLVVQNVMIDDAGRYTCEMSNPLGTERAHSQLSILPTPGCRKDGTTVG

SEQ ID NO: 4 - DNA, 2283 bp, Mus musculus
caggctggcccgcgggccccctgcgcggccgcctgcacttgcgccggggactcgctggactgcagtgggcgcgggctggcgacgctgccccgggacctgccctcctggacgcgcagcctaaacctgagttataacagactctccgagatcgactctgctgcttttgaggacttgacgaatctgcaggaagtgtacctcaacagcaatgagctgacagccataccatcactgggcgctgcttccataggagttgtctctctctttttgcagcacaacaagatccttagtgtggatgggagccagctgaagtcgtacctgtccttggaagtgctggatctgagttccaacaacatcacggaaattcggagctcctgtttcccgaacggcctgcgtataagggaactcaacttggcgagcaaccgcatcagcatcctggagtctggagcatttgatggtctgtcgcggtcactgctgactctccgtctgagcaaaaacaggatcacccagcttcctgtgaaagcgttcaagctacccaggctgacacaactagacctgaatcggaatcggattcggctgattgaaggcctcacgttccaggggctcgacagcttagaggtgctgaggcttcagaggaacaacatcagcaggctgacggacggggccttctgggggctgtctaagatgcacgtgctgcacctggagtacaacagtctggtggaagtgaacagtggctccctctatggcctcacagccctgcaccagctgcacctcagcaacaactccatctctcgaattcagcgtgatggctggagcttctgccaaaagctgcatgagttgattctgtccttcaacaacctcacgcggctggatgaggagagtctagcggagttgagcagcctcagtatcctgcgcctcagtcacaacgccatcagtcacattgctgaaggcgccttcaagggactcaagagtctgcgggtcttggacctggaccataacgagatctcgggtacaatcgaggataccagtggtgcctttacggggcttgacaacctcagcaagctgactctgtttggaaacaagatcaaatctgtggctaagagagccttctcgggcctggaaagcctggaacacctgaaccttggagagaatgcaatcaggtctgtccagtttgatgcctttgcaaagatgaagaaccttaaagagctctacatcagcagtgagagcttcctgtgtgactgccagctcaagtggctgcccccatggctaatgggtaggatgctgcaggcctttgtgacagccacctgtgcccatccagagtcgctgaagggccagagcattttctcagtgctgccagacagctttgtgtgtgatgactttccaaagccacagatcatcacccagcctgagacgaccatggctgtggtgggcaaggacatccgtttcacatgctccgcagccagcagcagcagctcaccaatgaccttcgcctggaagaaggacaatgaggtcctggccaatgcagacatggagaactttgcccacgtccgtgcacaggacggcgaagtgatggagtataccactatcctgcacctccgtcacgtcacctttgggcacgagggccgctaccagtgtatcatcacaaaccactttggctccacatactcccacaaagccaggctcactgtgaatgtgttgccatcattcactaaaataccccatgacattgccatccggactggcaccacagcccgcctcgagtgtgctgccacgggccaccctaaccctcagattgcctggcagaaggatggaggcaccgatttcccggcagctcgtgagcgacgcatgcatgttatgccagacgatgatgtgttcttcatcactgatgtgaaaatagacgacatgggggtctacagctgcactgcccagaactcggcaggctcggtttcagccaacgctaccctcacagtcttagaaactccatccttggcagtgcctctggaagaccgtgtggtaactgtgggagaaacagtggccttccagtgcaaagcaaccgggagccccacaccacgcatcacctggcttaagggaggtcgcccattgagcctcacagagcgccaccatttcactccaggcaaccagctgctggttgttcagaatgtgatgatagacgatgcagggcggtatacctgtgagatgtctaatcccctgggcactgagcgagcacatagccagctgagcattttacctacccctggctgccggaaggatgggaccaccgtaggc

SEQ ID NO: 5 - protein, 5 aa, Artificial Sequence
  Heavy chain CDR 1
NYAMS

SEQ ID NO: 6 - protein, 17 aa, Artificial Sequence
  Heavy chain CDR 2
VISHGGGSTYYADSVKG

SEQ ID NO: 7 - protein, 18 aa, Artificial Sequence
  Heavy chain CDR 3
VISNCHLGVCYYSNGMDV

SEQ ID NO: 8 - protein, 13 aa, Artificial Sequence
  Light chain CDR 1
SGSSSNIGDNYVS

SEQ ID NO: 9 - protein, 7 aa, Artificial Sequence
  Light chain CDR 2
DNNKRPS

SEQ ID NO: 10 - protein, 10 aa, Artificial Sequence
  Light chain CDR 3
WDGSLSAGRV

SEQ ID NO: 11 - protein, 127 aa, Artificial Sequence
  Heavy chain variable region
EVQLLESGGGLVQPGGSLRLSCAASGFTFSNYAMSWVRQAPGKGLEWVSVISHGGGSTYYADSVKGRFTISRDNSKNTLYLQMNSLRAEDTAVYYCARVISNCHLGVCYYSNGMDVWGQGTLVTVSS

SEQ ID NO: 12 - protein, 111 aa, Artificial Sequence
  Light chain variable region
QLVLTQPPSVSAAPGQRVSISCSGSSSNIGDNYVSWYQQVPGSAPKLLIYDNNKRPSGIPDRFSASKSGTSATLGITGLQTGDEADYYCATWDGSLSAGRVFGGGTKLTVL

SEQ ID NO: 13 - DNA, 15 bp, Artificial Sequence
  Heavy chain CDR 1
aactacgccatgagc

SEQ ID NO: 14 - DNA, 51 bp, Artificial Sequence
  Heavy chain CDR 2
gtgatctctcacggcggaggcagcacctactacgccgattctgtgaagggc

SEQ ID NO: 15 - DNA, 54 bp, Artificial Sequence
  Heavy chain CDR 3
gtgatcagcaactgccacctgggcgtgtgctactacagcaacggcatggatgtg

SEQ ID NO: 16 - DNA, 39 bp, Artificial Sequence
  Light chain CDR 1
agcggcagcagcagcaacatcggcgacaactacgtgtcc

SEQ ID NO: 17 - DNA, 21 bp, Artificial Sequence
  Light chain CDR 2
gacaacaacaagcggcccagc

SEQ ID NO: 18 - DNA, 30 bp, Artificial Sequence
  Light chain CDR 3
tgggatggctccctgagcgccggaagagtt

SEQ ID NO: 19 - DNA, 381 bp, Artificial Sequence
  Heavy chain variable region
gaagttcagctgcttgagtctggcggaggactggttcaacctggcggaagcctgagactgtcttgtgccgccagcggcttcaccttcagcaactacgccatgagctgggtccgacaggcccctggaaaaggccttgaatgggtgtccgtgatctctcacggcggaggcagcacctactacgccgattctgtgaagggcagattcaccatcagccgggacaacagcaagaacaccctgtacctgcagatgaacagcctgagagccgaggacaccgccgtgtactattgcgccagagtgatcagcaactgccacctgggcgtgtgctactacagcaacggcatggatgtgtggggccagggcacactggttaccgttagttct

SEQ ID NO: 20 - DNA, 333 bp, Artificial Sequence
  Light chain variable region
caactggttctgacacagcctccaagcgtgtcagctgcccctggacagagagtgtccatcagctgtagcggcagcagcagcaacatcggcgacaactacgtgtcctggtatcagcaggtcccaggctctgcccctaagctgctgatctacgacaacaacaagcggcccagcggcatccccgatagattttctgccagcaagagcggcaccagcgccacactgggaattacaggactgcagacaggcgacgaggccgactactattgtgccacatgggatggctccctgagcgccggaagagtttttggcggaggcaccaagctgaccgtgctt

SEQ ID NO: 21 - protein, 328 aa, Mus musculus
TTAPSVYPLAPVCGDTTGSSVTLGCLVKGYFPEPVTLTWNSGSLSSGVHTFPAVLQSDLYTLSSSVTVTSSTWPSQSITCNVAHPASSTKVDKKIEPRGPTIKPCPPCKCPAPNLLGGPSVFIFPPKIKDVLMISLSPIVTCVVVDVSEDDPDVQISWFVNNVEVHTAQTQTHREDYNSTLRVVSALPIQHQDWMSGKEFKCKVNNKDLPAPIERTISKPKGSVRAPQVYVLPPPEEEMTKKQVTLTCMVTDFMPEDIYVEWTNNGKTELNYKNTEPVLDSDGSYFMYSKLRVEKKNWVERNSYSCSVVHEGLHNHHTTKSFSRTPGK

SEQ ID NO: 22 - protein, 107 aa, Mus musculus
RTVAAPTVSIFPPSSEQLTSGGASVVCFLNNFYPKDINVKWKIDGSERQNGVLNSWTDQDSKDSTYSMSSTLTLTKDEYERHNSYTCEATHKTSTSPIVKSFNRNEC

SEQ ID NO: 23 - protein, 330 aa, Homo sapiens [sequence omitted]

SEQ ID NO: 24 - protein, 330 aa, Homo sapiens
ASTKGPSVFPLAPSSKSTSGGTAALGCLVKDYFPEPVTVSWNSGALTSGVHTFPAVLQSSGLYSLSSVVTVPSSSLGTQTYICNVNHKPSNTKVDKKVEPKSCDKTHTCPPCPAPELLGGPSVFLFPPKPKDTLMISRTPEVTCVVVDVSHEDPEVKFNWYVDGVEVHNAKTKPREEQYNSTYRVVSVLTVLHQDWLNGKEYKCKVSNKALPAPIEKTISKAKGQPREPQVYTLPPSREEMTKNQVSLTCLVKGFYPSDIAVEWESNGQPENNYKTTPPVLDSDGSFFLYSKLTVDKSRWQQGNVFSCSVMHEALHNHYTQKSLSLSPGK

SEQ ID NO: 25 - protein, 107 aa, Homo sapiens [sequence omitted]

SEQ ID NO: 26 - protein, 107 aa, Homo sapiens
RSVAAPSVFIFPPSDEQLKSGTASVVCLLNNFYPREAKVQWKVDNALQSGNSQESVTEQDSKDSTYSLSSTLTLSKADYEKHKVYACEVTHQGLSSPVTKSFNRGEC

SEQ ID NO: 27 - protein, 326 aa, Homo sapiens
ASTKGPSVFPLAPCSRSTSESTAALGCLVKDYFPEPVTVSWNSGALTSGVHTFPAVLQSSGLYSLSSVVTVPSSNFGTQTYTCNVDHKPSNTKVDKTVERKCCVECPPCPAPPVAGPSVFLFPPKPKDTLMISRTPEVTCVVVDVSHEDPEVQFNWYVDGVEVHNAKTKPREEQFNSTFRVVSVLTVVHQDWLNGKEYKCKVSNKGLPAPIEKTISKTKGQPREPQVYTLPPSREEMTKNQVSLTCLVKGFYPSDISVEWESNGQPENNYKTTPPMLDSDGSFFLYSKLTVDKSRWQQGNVFSCSVMHEALHNHYTQKSLSLSPGK

SEQ ID NO: 28 - protein, 377 aa, Homo sapiens
ASTKGPSVFPLAPCSRSTSGGTAALGCLVKDYFPEPVTVSWNSGALTSGVHTFPAVLQSSGLYSLSSVVTVPSSSLGTQTYTCNVNHKPSNTKVDKRVELKTPLGDTTHTCPRCPEPKSCDTPPPCPRCPEPKSCDTPPPCPRCPEPKSCDTPPPCPRCPAPELLGGPSVFLFPPKPKDTLMISRTPEVTCVVVDVSHEDPEVQFKWYVDGVEVHNAKTKPREEQYNSTFRVVSVLTVLHQDWLNGKEYKCKVSNKALPAPIEKTISKTKGQPREPQVYTLPPSREEMTKNQVSLTCLVKGFYPSDIAVEWESSGQPENNYNTTPPMLDSDGSFFLYSKLTVDKSRWQQGNIFSCSVMHEALHNRFTQKSLSLSPGK

SEQ ID NO: 29 - protein, 327 aa, Homo sapiens
ASTKGPSVFPLAPCSRSTSESTAALGCLVKDYFPEPVTVSWNSGALTSGVHTFPAVLQSSGLYSLSSVVTVPSSSLGTKTYTCNVDHKPSNTKVDKRVESKYGPPCPSCPAPEFLGGPSVFLFPPKPKDTLMISRTPEVTCVVVDVSQEDPEVQFNWYVDGVEVHNAKTKPREEQFNSTYRVVSVLTVLHQDWLNGKEYKCKVSNKGLPSSIEKTISKAKGQPREPQVYTLPPSQEEMTKNQVSLTCLVKGFYPSDIAVEWESNGQPENNYKTTPPVLDSDGSFFLYSRLTVDKSRWQEGNVFSCSVMHEALHNHYTQKSLSLSLGK

SEQ ID NO: 30 - protein, 332 aa, Artificial Sequence
  Heavy chain constant region
ASAKTTAPSVYPLAPVCGDTTGSSVTLGCLVKGYFPEPVTLTWNSGSLSSGVHTFPAVLQSDLYTLSSSVTVTSSTWPSQSITCNVAHPASSTKVDKKIEPRGPTIKPCPPCKCPAPNLLGGPSVFIFPPKIKDVLMISLSPIVTCVVVDVSEDDPDVQISWFVNNVEVHTAQTQTHREDYNSTLRVVSALPIQHQDWMSGKEFKCKVNNKDLPAPIERTISKPKGSVRAPQVYVLPPPEEEMTKKQVTLTCMVTDFMPEDIYVEWTNNGKTELNYKNTEPVLDSDGSYFMYSKLRVEKKNWVERNSYSCSVVHEGLHNHHTTKSFSRTPGK

SEQ ID NO: 31 - protein, 107 aa, Artificial Sequence
  Light chain constant region
RTDAAPTVSIFPPSSEQLTSGGASVVCFLNNFYPKDINVKWKIDGSERQNGVLNSWTDQDSKDSTYSMSSTLTLTKDEYERHNSYTCEATHKTSTSPIVKSFNRNEC

SEQ ID NO: 32 - protein, 245 aa, Artificial Sequence
  Hybrid Fc Heavy region
RNTGRGGEEKKKEKEKEEQEERETKTPECPSHTQPLGVFLFPPKPKDTLMISRTPEVTCVVVDVSQEDPEVQFNWYVDGVEVHNAKTKPREEQFNSTYRVVSVLTVLHQDWLNGKEYKCKVSNKGLPSSIEKTISKAKGQPREPQVYTLPPSQEEMTKNQVSLTCLVKGFYPSDIAVEWESNGQPENNYKTTPPVLDSDGSFFLYSRLTVDKSRWQEGNVFSCSVMHEALHNHYTQKSLSLSLGK

SEQ ID NO: 33 - DNA, 990 bp, Homo sapiens
gctagcaccaagggcccatcggtcttccccctggcgccctcctccaagagcacctctgggggcacagcggccctgggctgcctggtcaaggactacttccccgaaccggtgacggtgtcgtggaactcaggggccctgaccagcggcgtgcacaccttcccggctgtcctacagtcctcaggactctactccctcagcagcgtggtgaccgtgccctccagcagcctgggcacccagacctacatctgcaacgtgaatcacaagcccagcaacaccaaggtggacaagaaagttgagcccaaatcttgtgacaaaactcacacatgcccaccgtgcccagcacctgaactcctggggggaccgtcagtcttcctcttccccccaaaacccaaggacaccctcatgatctcccggacccctgaggtcacatgcgtggtggtggacgtgagccacgaagaccctgaggtcaagttcaactggtacgtggacggcgtggaggtgcataatgccaagacaaagccgcgggaggagcagtacaacagcacgtaccgtgtggtcagcgtcctcaccgtcctgcaccaggactggctgaatggcaaggagtacaagtgcaaggtctccaacaaagccctcccagcccccatcgagaaaaccatctccaaagccaaagggcagccccgagaaccacaggtgtacaccctgcccccatcccgggaggagatgaccaagaaccaggtcagcctgacctgcctggtcaaaggcttctatcccagcgacatcgccgtggagtgggagagcaatgggcagccggagaacaactacaagaccacgcctcccgtgctggactccgacggctccttcttcctctacagcaagctcaccgtggacaagagcaggtggcagcaggggaacgtcttctcatgctccgtgatgcatgaggctctgcacaaccactacacgcagaagagcctctccctgtctccgggtaaa

SEQ ID NO: 34 - DNA, 321 bp, Homo sapiens
agatctgtggctgcaccatctgtcttcatcttcccgccatctgatgagcagttgaaatctggaactgcctctgttgtgtgcctgctgaataacttctatcccagagaggccaaagtacagtggaaggtggataacgccctccaatcgggtaactcccaggagagtgtcacagagcaggacagcaaggacagcacctacagcctcagcagcaccctgacgctgagcaaagcagactacgagaaacacaaagtctacgcctgcgaagtcacccatcagggcctgagctcgcccgtcacaaagagcttcaacaggggagagtgt

SEQ ID NO: 35 - DNA, 999 bp, Artificial Sequence
  Heavy chain constant region
gctagcgccaaaacaacagccccctccgtataccccctagcccccgtatgcggcgacaccaccggctcctccgtaaccctaggctgcctagtaaaaggctacttccccgaacccgtaaccctaacctggaactccggctccctatcctccggcgtacacaccttccccgccgtactacaatccgacctatacaccctatcctcctccgtaaccgtaacctcctccacctggccctcccaatccatcacctgcaacgtagcccaccccgcctcctccaccaaagtagacaaaaaaatcgagccaaggggccccaccatcaagccttgccctccctgcaagtgccctgcccccaacctgctgggcggcccctccgtgttcatcttccctccaaagatcaaggacgtgctgatgatctccctgagccccatcgtgacctgcgtggtggtggacgtgtccgaggacgaccctgacgtgcagatcagctggttcgtgaacaacgtggaggtgcacaccgcccagacccagacccacagagaggactacaactccaccctgagggtggtgagcgccctgccaatccagcaccaggactggatgtccggcaaggagttcaagtgcaaggtgaacaacaaggacctgccagccccaatcgagaggaccatcagcaagcctaagggctccgtgagggccccccaggtgtacgtgctgccccctcctgaggaggagatgaccaagaagcaggtgaccctgacctgcatggtgaccgacttcatgcctgaggacatctacgtggagtggaccaacaacggcaagaccgagctgaactacaagaacaccgagcctgtgctggacagcgacggcagctacttcatgtacagcaagctgagggtggagaagaagaactgggtggagagaaactcctactcctgctccgtggtgcacgagggcctgcacaaccaccacaccaccaagagcttctccagaacccccgggaagtga

SEQ ID NO: 36 - DNA, 321 bp, Artificial Sequence
  Light chain constant region
cgtacggatgctgcaccaactgtatccatcttcccaccatccagtgagcagttaacatctggaggtgcctcagtcgtgtgcttcttgaacaacttctaccccaaagacatcaatgtcaagtggaagattgatggcagtgaacgacaaaatggcgtcctgaacagttggactgatcaggacagcaaagacagcacctacagcatgagcagcaccctcacgttgaccaaggacgagtatgaacgacataacagctatacctgtgaggccactcacaagacatcaacttcacccattgtcaagagcttcaacaggaatgagtgt

SEQ ID NO: 37 - protein, 457 aa, Artificial Sequence
  Heavy chain
EVQLLESGGGLVQPGGSLRLSCAASGFTFSNYAMSWVRQAPGKGLEWVSVISHGGGSTYYADSVKGRFTISRDNSKNTLYLQMNSLRAEDTAVYYCARVISNCHLGVCYYSNGMDVWGQGTLVTVSSAKTTAPSVYPLAPVCGDTTGSSVTLGCLVKGYFPEPVTLTWNSGSLSSGVHTFPAVLQSDLYTLSSSVTVTSSTWPSQSITCNVAHPASSTKVDKKIEPRGPTIKPCPPCKCPAPNLLGGPSVFIFPPKIKDVLMISLSPIVTCVVVDVSEDDPDVQISWFVNNVEVHTAQTQTHREDYNSTLRVVSALPIQHQDWMSGKEFKCKVNNKDLPAPIERTISKPKGSVRAPQVYVLPPPEEEMTKKQVTLTCMVTDFMPEDIYVEWTNNGKTELNYKNTEPVLDSDGSYFMYSKLRVEKKNWVERNSYSCSVVHEGLHNHHTTKSFSRTPGK

SEQ ID NO: 38 - protein, 457 aa, Artificial Sequence
  Heavy chain
EVQLLESGGGLVQPGGSLRLSCAASGFTFSNYAMSWVRQAPGKGLEWVSVISHGGGSTYYADSVKGRFTISRDNSKNTLYLQMNSLRAEDTAVYYCARVISNCHLGVCYYSNGMDVWGQGTLVTVSSASTKGPSVFPLAPSSKSTSGGTAALGCLVKDYFPEPVTVSWNSGALTSGVHTFPAVLQSSGLYSLSSVVTVPSSSLGTQTYICNVNHKPSNTKVDKKVEPKSCDKTHTCPPCPAPELLGGPSVFLFPPKPKDTLMISRTPEVTCVVVDVSHEDPEVKFNWYVDGVEVHNAKTKPREEQYNSTYRVVSVLTVLHQDWLNGKEYKCKVSNKALPAPIEKTISKAKGQPREPQVYTLPPSREEMTKNQVSLTCLVKGFYPSDIAVEWESNGQPENNYKTTPPVLDSDGSFFLYSKLTVDKSRWQQGNVFSCSVMHEALHNHYTQKSLSLSPGK

SEQ ID NO: 39 - protein, 218 aa, Artificial Sequence
  Light chain
QLVLTQPPSVSAAPGQRVSISCSGSSSNIGDNYVSWYQQVPGSAPKLLIYDNNKRPSGIPDRFSASKSGTSATLGITGLQTGDEADYYCATWDGSLSAGRVFGGGTKLTVLRADAAPTVSIFPPSSEQLTSGGASVVCFLNNFYPKDINVKWKIDGSERQNGVLNSWTDQDSKDSTYSMSSTLTLTKDEYERHNSYTCEATHKTSTSPIVKSFNRNEC

SEQ ID NO: 40 - protein, 218 aa, Artificial Sequence
  Light chain
QLVLTQPPSVSAAPGQRVSISCSGSSSNIGDNYVSWYQQVPGSAPKLLIYDNNKRPSGIPDRFSASKSGTSATLGITGLQTGDEADYYCATWDGSLSAGRVFGGGTKLTVLRTVAAPSVFIFPPSDEQLKSGTASVVCLLNNFYPREAKVQWKVDNALQSGNSQESVTEQDSKDSTYSLSSTLTLSKADYEKHKVYACEVTHQGLSSPVTKSFNRGEC

SEQ ID NO: 41 - DNA, 1380 bp, Artificial Sequence
  Heavy chain
gaagttcagctgcttgagtctggcggaggactggttcaacctggcggaagcctgagactgtcttgtgccgccagcggcttcaccttcagcaactacgccatgagctgggtccgacaggcccctggaaaaggccttgaatgggtgtccgtgatctctcacggcggaggcagcacctactacgccgattctgtgaagggcagattcaccatcagccgggacaacagcaagaacaccctgtacctgcagatgaacagcctgagagccgaggacaccgccgtgtactattgcgccagagtgatcagcaactgccacctgggcgtgtgctactacagcaacggcatggatgtgtggggccagggcacactggttaccgttagttctgctagcgccaaaacaacagccccctccgtataccccctagcccccgtatgcggcgacaccaccggctcctccgtaaccctaggctgcctagtaaaaggctacttccccgaacccgtaaccctaacctggaactccggctccctatcctccggcgtacacaccttccccgccgtactacaatccgacctatacaccctatcctcctccgtaaccgtaacctcctccacctggccctcccaatccatcacctgcaacgtagcccaccccgcctcctccaccaaagtagacaaaaaaatcgagccaaggggccccaccatcaagccttgccctccctgcaagtgccctgcccccaacctgctgggcggcccctccgtgttcatcttccctccaaagatcaaggacgtgctgatgatctccctgagccccatcgtgacctgcgtggtggtggacgtgtccgaggacgaccctgacgtgcagatcagctggttcgtgaacaacgtggaggtgcacaccgcccagacccagacccacagagaggactacaactccaccctgagggtggtgagcgccctgccaatccagcaccaggactggatgtccggcaaggagttcaagtgcaaggtgaacaacaaggacctgccagccccaatcgagaggaccatcagcaagcctaagggctccgtgagggccccccaggtgtacgtgctgccccctcctgaggaggagatgaccaagaagcaggtgaccctgacctgcatggtgaccgacttcatgcctgaggacatctacgtggagtggaccaacaacggcaagaccgagctgaactacaagaacaccgagcctgtgctggacagcgacggcagctacttcatgtacagcaagctgagggtggagaagaagaactgggtggagagaaactcctactcctgctccgtggtgcacgagggcctgcacaaccaccacaccaccaagagcttctccagaacccccgggaagtga

SEQ ID NO: 42 - DNA, 1371 bp, Artificial Sequence
  Heavy chain
gaagttcagctgcttgagtctggcggaggactggttcaacctggcggaagcctgagactgtcttgtgccgccagcggcttcaccttcagcaactacgccatgagctgggtccgacaggcccctggaaaaggccttgaatgggtgtccgtgatctctcacggcggaggcagcacctactacgccgattctgtgaagggcagattcaccatcagccgggacaacagcaagaacaccctgtacctgcagatgaacagcctgagagccgaggacaccgccgtgtactattgcgccagagtgatcagcaactgccacctgggcgtgtgctactacagcaacggcatggatgtgtggggccagggcacactggttaccgttagttctgctagcaccaagggcccatcggtcttccccctggcgccctcctccaagagcacctctgggggcacagcggccctgggctgcctggtcaaggactacttccccgaaccggtgacggtgtcgtggaactcaggggccctgaccagcggcgtgcacaccttcccggctgtcctacagtcctcaggactctactccctcagcagcgtggtgaccgtgccctccagcagcctgggcacccagacctacatctgcaacgtgaatcacaagcccagcaacaccaaggtggacaagaaagttgagcccaaatcttgtgacaaaactcacacatgcccaccgtgcccagcacctgaactcctggggggaccgtcagtcttcctcttccccccaaaacccaaggacaccctcatgatctcccggacccctgaggtcacatgcgtggtggtggacgtgagccacgaagaccctgaggtcaagttcaactggtacgtggacggcgtggaggtgcataatgccaagacaaagccgcgggaggagcagtacaacagcacgtaccgtgtggtcagcgtcctcaccgtcctgcaccaggactggctgaatggcaaggagtacaagtgcaaggtctccaacaaagccctcccagcccccatcgagaaaaccatctccaaagccaaagggcagccccgagaaccacaggtgtacaccctgcccccatcccgggaggagatgaccaagaaccaggtcagcctgacctgcctggtcaaaggcttctatcccagcgacatcgccgtggagtgggagagcaatgggcagccggagaacaactacaagaccacgcctcccgtgctggactccgacggctccttcttcctctacagcaagctcaccgtggacaagagcaggtggcagcaggggaacgtcttctcatgctccgtgatgcatgaggctctgcacaaccactacacgcagaagagcctctccctgtctccgggtaaa

SEQ ID NO: 43 - DNA, 654 bp, Artificial Sequence
  Light chain
caactggttctgacacagcctccaagcgtgtcagctgcccctggacagagagtgtccatcagctgtagcggcagcagcagcaacatcggcgacaactacgtgtcctggtatcagcaggtcccaggctctgcccctaagctgctgatctacgacaacaacaagcggcccagcggcatccccgatagattttctgccagcaagagcggcaccagcgccacactgggaattacaggactgcagacaggcgacgaggccgactactattgtgccacatgggatggctccctgagcgccggaagagtttttggcggaggcaccaagctgaccgtgcttcgtacggatgctgcaccaactgtatccatcttcccaccatccagtgagcagttaacatctggaggtgcctcagtcgtgtgcttcttgaacaacttctaccccaaagacatcaatgtcaagtggaagattgatggcagtgaacgacaaaatggcgtcctgaacagttggactgatcaggacagcaaagacagcacctacagcatgagcagcaccctcacgttgaccaaggacgagtatgaacgacataacagctatacctgtgaggccactcacaagacatcaacttcacccattgtcaagagcttcaacaggaatgagtgt

SEQ ID NO: 44 - DNA, 654 bp, Artificial Sequence
  Light chain
caactggttctgacacagcctccaagcgtgtcagctgcccctggacagagagtgtccatcagctgtagcggcagcagcagcaacatcggcgacaactacgtgtcctggtatcagcaggtcccaggctctgcccctaagctgctgatctacgacaacaacaagcggcccagcggcatccccgatagattttctgccagcaagagcggcaccagcgccacactgggaattacaggactgcagacaggcgacgaggccgactactattgtgccacatgggatggctccctgagcgccggaagagtttttggcggaggcaccaagctgaccgtgcttagatctgtggctgcaccatctgtcttcatcttcccgccatctgatgagcagttgaaatctggaactgcctctgttgtgtgcctgctgaataacttctatcccagagaggccaaagtacagtggaaggtggataacgccctccaatcgggtaactcccaggagagtgtcacagagcaggacagcaaggacagcacctacagcctcagcagcaccctgacgctgagcaaagcagactacgagaaacacaaagtctacgcctgcgaagtcacccatcagggcctgagctcgcccgtcacaaagagcttcaacaggggagagtgt

SEQ ID NO: 45 - DNA, 24 bp, Artificial Sequence
  mouse Lrig-1 forward primer
gacggaattcagtgaggagaacct

SEQ ID NO: 46 - DNA, 24 bp, Artificial Sequence
  mouse Lrig-1 reverse primer
caactggtagtggcagcttgtagg

SEQ ID NO: 47 - DNA, 24 bp, Artificial Sequence
  mouse Lrig-2 forward primer
tcacaaggaacattgtctgaacca

SEQ ID NO: 48 - DNA, 24 bp, Artificial Sequence
  mouse Lrig-2 reverse primer
gcctgatctaacacatcctcctca

SEQ ID NO: 49 - DNA, 24 bp, Artificial Sequence
  mouse Lrig-3 forward primer
cagcaccttgagctgaacagaaac

SEQ ID NO: 50 - DNA, 24 bp, Artificial Sequence
  mouse Lrig-3 reverse primer
ccagcctttggtaatctcggttag

SEQ ID NO: 51 - DNA, 24 bp, Artificial Sequence
  mouse FOXP3 forward primer
ctttcacctatcccacccttatcc

SEQ ID NO: 52 - DNA, 24 bp, Artificial Sequence
  mouse FOXP3 reverse primer
attcatctacggtccacactgctc

SEQ ID NO: 53 - DNA, 20 bp, Artificial Sequence
  ACTG1 forward primer
ggcgtcatggtgggcatggg

SEQ ID NO: 54 - DNA, 20 bp, Artificial Sequence
  ACTG1 reverse primer
atggcgtggggaagggcgta